European Patent Specification EP 3 223 835 B1, published November 13, 2024. Title: Intestinal Microbiota and GVHD. Applicant: van den Brink, Marcel Jenq, Robert Pamer, Eric G Taur, Ying Shono, Yusuke. The sequence listing filed with the application follows.

SEQUENCE LISTING (18 sequences)

SEQ ID NO: 1 - DNA, 331 bp, Ruminococcus obeum
agcgtagacggattagcaagtctgatgtgaaaggcaggggctcaacccctggactgcattggaaactgccagtcttgagtgccggagaggtaagcggaattcctagtgtagcggtgaaatgcgtagatattaggaggaacaccagtggcgaaggcggcttactggacggcaactgacgttgaggctcgaaagcgtggggagcaaacaggattagataccctggtagtccacgccgtaaacgatgaatactaggtgttggggagcaaagctcttcggtgccgccgcaaacgcattaagtattccacctggggagtacgttcgcaagaatgaa

SEQ ID NO: 2 - DNA, 333 bp, Bifidobacterium dentium
ctcgtaggcggttcgtcgcgtccggtgtgaaagcccatcgcttaacggtgggtctgcgccgggtacgggcgggctggagtgcggtaggggagactggaattcccggtgtaacggtggaatgtgtagatatcgggaagaacaccaatggcgaaggcaggtctctgggccgtcactgacgctgaggagcgaaagcgtggggagcgaacaggattagataccctggtagtccacgccgtaaacggtggatgctggatgtggggcccgttccacgggttccgtgtcggagccaacgcgttaagcatcccgcctggggagtatgcacgcaagtgtgaa

SEQ ID NO: 3 - DNA, 331 bp, Clostridium hathewayi
agcgcaggcggtttgataagtctgaagtgaaagcccggggcacaaccccggtactgctttggaaactgttagacttgagtgcaggagaggtaagtggaattcctagtgtagcggtgaaatgcgtagatattaggaggaacaccagtggcgaaggcggcttactggactgtaactgacgttgaggctcgaaagcgtggggagcaaacaggattagataccctggtagtccacgctgtaaacgatgaatactaggtgtcggggggcaaagcccttcggtgccgccgcaaacgcaataagtattccacctggggagtacgttcgcaagaatgaa

SEQ ID NO: 4 - DNA, 332 bp, Eubacterium desmolans
cgagtaggcgggctggcaagttgggagtgaaatcccggggcttaaccccggaactgctttcaaaactgctggtcttgagtgatggagaggcaggcggaattccgtgtgtagcggtgaaatgcgtagatatacggaggaacaccagtggcgaaggcggcctgctggacattaactgacgctgaggagcgaaagcgtggggagcaaacaggattagataccctggtagtccacgccgtaaacgatggatactaggtgtgggaggtattgaccccttccgtgccggagttaacacaataagtatcccacctggggagtacggccgcaaggttgaa

SEQ ID NO: 5 - DNA, 331 bp, Dorea longicatena
agcgtagacggcacggcaagccagatgtgaaagcccggggctcaaccccgggactgcatttggaactgctgagctagagtgtcggagaggcaagtggaattcctagtgtagcggtgaaatgcgtagatattaggaggaacaccagtggcgaaggcggcttgctggacgatgactgacgttgaggctcgaaagcgtggggagcaaacaggattagataccctggtagtccacgccgtaaacgatgactgctaggtgtcgggtggcaaagccattcggtgccgcagctaacgcaataagcagtccacctggggagtacgttcgcaagaatgaa

SEQ ID NO: 6 - DNA, 331 bp, Lactococcus raffinolactis
agcgcaggtggtttaataagtctgatgtaaaaggcagtggctcaaccattgtgtgcattggaaactgttagacttgagtgcagtagaggagagtggaattccatgtgtagcggtgaaatgcgtagatatatggaggaacaccggtggcgaaagcggctctctggactgtcactgacactgaggctcgaaagcgtgggtagcaaacaggattagataccctggtagtccacgccgtaaacgatgagtgctagttgtttggggctatccagccctaagtgacgcagcaaacgcattaagcactccgcctggggagtacgaccgcaaggttgaa

SEQ ID NO: 7 - DNA, 331 bp, Ruminococcus faecis
agcgtagacggagcagcaagtctgatgtgaaaacccggggctcaaccgcgggactgcattggaaactgttgatctggagtgccggagaggtaagcggaattcctagtgtagcggtgaaatgcgtagatattaggaggaacaccagtggcgaaggcggcttactggacggtaactgacgttgaggctcgaaagcgtggggagcaaacaggattagataccctggtagtccacgccgtaaacgatgactactaggtgtcgggtggcaaagccattcggtgccgcagccaacgcaataagtagtccacctggggagtacgttcgcaagaatgaa

SEQ ID NO: 8 - DNA, 331 bp, Eubacterium contortum
agcgtaggcggttatgcaagtcagatgtgaaagcccggggcttaaccccgggactgcatttgaaactgtgtaactagagtgtcggagagggaagtggaattcctagtgtagcggtgaaatgcgtagatattaggaggaacaccagtggcgaaggcggcttactggacgataactgacgctgaggctcgaaagcgtggggagcaaacaggattagataccctggtagtccacgccgtaaacgatgaatactaggtgttggggagcaaagctcttcggtgccgcagcaaacgcaataagtattccacctggggagtacgttcgcaagaatgaa

SEQ ID NO: 9 - DNA, 331 bp, Ruminococcus faecis
agcgtagacggaatggcaagtctgatgtgaaaggccggggctcaaccccgggactgcattggaaactgtcaatctagagtaccggaggggtaagtggaattcctagtgtagcggtgaaatgcgtagatattaggaggaacaccagtggcgaaggcggcttactggacggtaactgacgttgaggctcgaaagcgtggggagcaaacaggattagataccctggtagtccacgccgtaaacgatgaatactaggtgttggggagcaaagctcttcggtgccgcagcaaacgcaataagtattccacctggggagtacgttcgcaagaatgaa

SEQ ID NO: 10 - DNA, 332 bp, Lactobacillus parafarraginis
agcgcaggcggttttttaggtctgatgtgaaagccttcggcttaaccggagaagggcatcggaaaccgggagacttgagtgcagaagaggacagtggaactccatgtgtagcggtgaaatgcgtagatatatggaagaacaccagtggcgaaggcggctgtctggtctgtaactgacgctgaggctcgaaagcatgggtagcgaacaggattagataccctggtagtccatgccgtaaacgatgagtgctaagtgttggagggtttccgcccttcagtgctgcagctaacgcattaagcactccgcctggggagtacgaccgcaaggttgaa

SEQ ID NO: 11 - DNA, 332 bp, Lactobacillus reuteri
agcgcaggcggttgcttaggtctgatgtgaaagccttcggcttaaccgaagaagtgcatcggaaaccgggcgacttgagtgcagaagaggacagtggaactccatgtgtagcggtggaatgcgtagatatatggaagaacaccagtggcgaaggcggctgtctggtctgcaactgacgctgaggctcgaaagcatgggtagcgaacaggattagataccctggtagtccatgccgtaaacgatgagtgctaggtgttggagggtttccgcccttcagtgccggagctaacgcattaagcactccgcctggggagtacgaccgcaaggttgaa

SEQ ID NO: 12 - DNA, 323 bp, Holdemania filiformis
tgcgcaggcggtttgttaagtttaaggtgaaagcgtggggcttaaccccatatagccttagaaactgacagactagagtacaggagagggcaatggaattccatgtgtagcggtaaaatgcgtagatatatggaggaacaccagtggcgaaggcggttgcctggcctgtaactgacgctcatgcacgaaagcgtggggagcaaataggattagataccctagtagtccacgccgtaaacgatgagaactaagtgttggggaaactcagtgctgcagttaacgcaataagttctccgcctggggagtatgcacgcaagtgtgaa

SEQ ID NO: 13 - DNA, 331 bp, Acidaminococcus intestini
catgtaggcgggcttttaagtctgacgtgaaaatgcggggcttaaccccgtatggcgttggatactggaagtcttgagtgcaggagaggaaaggggaattcccagtgtagcggtgaaatgcgtagatattgggaggaacaccagtggcgaaggcgcctttctggactgtgtctgacgctgagatgcgaaagccagggtagcaaacgggattagataccccggtagtcctggccgtaaacgatggatactaggtgtaggaggtatcgaccccttctgtgccggagttaacgcaataagtatcccgcctggggactacgatcgcaagattgaa

SEQ ID NO: 14 - DNA, 327 bp, Eubacterium biforme
tgcgtaggtggcagatcaagtctggagtaaaaggtatgggctcaacccgtactggctctggaaactgatcagctagagaacagaagaggacggcggaactccatgtgtagcggtaaaatgcgtagatatatggaagaacaccggtggcgaaggcggccgtctggtctggattctgacactgaagcacgaaagcgtggggagcaaataggattagataccctagtagtccacgccgtaaacgatgagaactaggtgttgggggaataactcagtgccgcagttaacgcagtaagttctccgcctggggagtacgttcgcaagaatgaa

SEQ ID NO: 15 - DNA, 329 bp, Clostridium sordellii
tgcgtaggcggtctttcaagccagaagtgaaaggctacggctcaaccgtagtaagcttttggaactgtaggacttgagtgcaggagaggagagtggaattcctagtgtagcggtgaaatgcgtagatattaggaggaacaccagtagcgaaggcggctctctggactgtaactgacgctgaggcacgaaagcgtggggagcaaacaggattagataccctggtagtccacgccgtaaacgatgagtactaggtgtcgggggttacccccctcggtgccgcagctaacgcattaagtactccgcctggggagtacgaccgcaaggttgaa

SEQ ID NO: 16 - DNA, 331 bp, Serratia fonticola
cacgcaggcggtttgttaagtcagatgtgaaatccccgagcttaacttgggaactgcatttgaaactggcaagctagagtcttgtagaggggggtagaattccaggtgtagcggggaaatgcgtagagatctggaggaataccggtggcgaaggcggccccctggacaaagactgacgctcaggtgcgaaagcgtggggagcaaacaggattagataccctggtagtccacgctgtaaacgatgtcgacttggaggttgtgcccttgaggcgtggcttccggagctaacgcgttaagtcgaccgcctggggagtacggccgcaaggttaaa

SEQ ID NO: 17 - DNA, 20 bp, Artificial Sequence
  SYNTHETIC OLIGONUCLEOTIDE
agagtttgatcctggctcag

SEQ ID NO: 18 - DNA, 19 bp, Artificial Sequence
  synthetic nucleotide
tgctgcctcccgtaggagt